European Patent Application EP 4 356 756 A1, published April 24, 2024. Title: Composition for preventing, improving, or treating degenerative arthritis comprising steamed ginger extract or 1-dehydro-6-gingerdione isolated therefrom as an active ingredient. Applicant: GENENCELL CO., LTD. The sequence listing filed with the application follows.

SEQUENCE LISTING (20 sequences)

SEQ ID NO: 1 - DNA, 22 bp, Artificial Sequence
  IL-1beta sense primer
gcaactgttcctgaactcaact

SEQ ID NO: 2 - DNA, 21 bp, Artificial Sequence
  IL-1beta antisense primer
atcttttggggtccgtcaact

SEQ ID NO: 3 - DNA, 19 bp, Artificial Sequence
  beta-actin sense primer
cgtgaaaagatgaccagat

SEQ ID NO: 4 - DNA, 18 bp, Artificial Sequence
  beta-actin antisense primer
accctcatagatggcaca

SEQ ID NO: 5 - DNA, 27 bp, Artificial Sequence
  IL-1beta sense primer
cacctctcaagcagagcacagcacctc

SEQ ID NO: 6 - DNA, 21 bp, Artificial Sequence
  IL-1beta antisense primer
gggttccatggtgaagtcaac

SEQ ID NO: 7 - DNA, 23 bp, Artificial Sequence
  TNF-alpha sense primer
tcgtctactactcctcagagccc

SEQ ID NO: 8 - DNA, 20 bp, Artificial Sequence
  TNF-alpha antisense primer
acttcagcgtctcgtgtgtt

SEQ ID NO: 9 - DNA, 20 bp, Artificial Sequence
  IFN-gamma sense primer
gcaaaggacggtaacacgaa

SEQ ID NO: 10 - DNA, 25 bp, Artificial Sequence
  IFN-gamma antisense primer
atggcctggttgttgtctttcaaga

SEQ ID NO: 11 - DNA, 20 bp, Artificial Sequence
  beta-actin sense primer
cgtgaaaagatgacccagat

SEQ ID NO: 12 - DNA, 19 bp, Artificial Sequence
  beta-actin antisense primer
accctcatagatgggcaca

SEQ ID NO: 13 - DNA, 19 bp, Artificial Sequence
  MMP-9 sense primer
agccgggaacgtatctgga

SEQ ID NO: 14 - DNA, 21 bp, Artificial Sequence
  MMP-9 antisense primer
tggaaactcacacgccagaag

SEQ ID NO: 15 - DNA, 20 bp, Artificial Sequence
  TIMP-1 sense primer
catctctggcctctggcatc

SEQ ID NO: 16 - DNA, 25 bp, Artificial Sequence
  TIMP-1 antisense primer
cataacgctggtataaggtggtctc

SEQ ID NO: 17 - DNA, 22 bp, Artificial Sequence
  TIMP-2 sense primer
ctgtgacccagtccatccagag

SEQ ID NO: 18 - DNA, 22 bp, Artificial Sequence
  TIMP-2 antisense primer
gacacgcttagcatcacccaga

SEQ ID NO: 19 - DNA, 20 bp, Artificial Sequence
  COL2 sense primer
ctgagggctcccagaacatc

SEQ ID NO: 20 - DNA, 20 bp, Artificial Sequence
  COL2 antisense primer
ttcgtccaggtaggcaatgc